European Patent Application EP 4 703 388 A1, published March 4, 2026. Title: 抗hTF抗体和抗hTF抗体-药物偶联物及其医药用途. Applicant: 江苏恒瑞医药股份有限公司. Application CN. The sequence listing filed with the application follows.

SEQUENCE LISTING (171 sequences)

SEQ ID NO: 1 - protein, 295 aa, Homo sapiens [sequence omitted]

SEQ ID NO: 2 - protein, 296 aa, Macaca fascicularis
  CHAIN 1..296: note = Cyno TF
METPAWPRVPRPETAVARTLLLGWVFAQVAGASGTTNTVAAYNLTWKSTNFKTILEWEPKPINQVYTVQISTKSGDWKSKCFYTADTECDLTDEIVKDVKQTYLARVFSYPAGHVESTGSTEEPPYENSPEFTPYLETNLGQPTIQSFEQVGTKVNVTVQDEWTLVRRNDTFLSLRDVFGKDLIYTLYYWKSSSSGKKTAKTNTNEFLIDVDKGENYCFSVQAVIPSRRTANRKSTDSPVECMGHEKGESREIFYIIGAVVFVVIILVIILAISLHKCKKARVGRSWKENSPLNVA

SEQ ID NO: 3 - protein, 295 aa, Rattus norvegicus
  CHAIN 1..295: note = Rat TF
MAIPMRPRLLAALAPTFLGFLLLQVAVGAGTPPGKAFNLTWISTDFKTILEWQPKPTNYTYTVQISDRSRNWKYKCTGTTDTECDLTDEIVKDVNWTYEARVLSVPWRNSTHGKETLFGTHGEEPPFTNARKFLPYRDTKIGQPVIQKYEQGGTKLKVTVKDSFTLVRKNGTFLTLRQVFGNDLGYILTYRKDSSTGRKTNTTHTNEFLIDVEKGVSYCFFAQAVIFSRKTNHKSPESITKCTEQWKSVLGETLIIVGAVVFLVTVFIILLTISLCKRRKNRAGQKRKNTPSRLA

SEQ ID NO: 4 - protein, 294 aa, Mus musculus
  CHAIN 1..294: note = Mouse TF
MAILVRPRLLAALAPTFLGCLLLQVIAGAGIPEKAFNLTWISTDFKTILEWQPKPTNYTYTVQISDRSRNWKNKCFSTTDTECDLTDEIVKDVTWAYEAKVLSVPRRNSVHGDGDQLVIHGEEPPFTNAPKFLPYRDTNLGQPVIQQFEQDGRKLNVVVKDSLTLVRKNGTFLTLRQVFGKDLGYIITYRKGSSTGKKTNITNTNEFSIDVEEGVSYCFFVQAMIFSRKTNQNSPGSSTVCTEQWKSFLGETLIIVGAVVLLATIFIILLSISLCKRRKNRAGQKGKNTPSRLA

SEQ ID NO: 5 - protein, 227 aa, synthetic construct
  CHAIN 1..227: note = hTF-his
SGTTNTVAAYNLTWKSTNFKTILEWEPKPVNQVYTVQISTKSGDWKSKCFYTTDTECDLTDEIVKDVKQTYLARVFSYPAGNVESTGSAGEPLYENSPEFTPYLETNLGQPTIQSFEQVGTKVNVTVEDERTLVRRNNTFLSLRDVFGKDLIYTLYYWKSSSSGKKTAKTNTNEFLIDVDKGENYCFSVQAVIPSRTVNRKSTDSPVECMGQEKGEFRETGHHHHHH

SEQ ID NO: 6 - protein, 451 aa, synthetic construct
  CHAIN 1..451: note = hTF-hFc
SGTTNTVAAYNLTWKSTNFKTILEWEPKPVNQVYTVQISTKSGDWKSKCFYTTDTECDLTDEIVKDVKQTYLARVFSYPAGNVESTGSAGEPLYENSPEFTPYLETNLGQPTIQSFEQVGTKVNVTVEDERTLVRRNNTFLSLRDVFGKDLIYTLYYWKSSSSGKKTAKTNTNEFLIDVDKGENYCFSVQAVIPSRTVNRKSTDSPVECMGQEKGEFREEPKSSDKTHTCPPCPAPELLGGPSVFLFPPKPKDTLMISRTPEVTCVVVDVSHEDPEVKFNWYVDGVEVHNAKTKPREEQYNSTYRVVSVLTVLHQDWLNGKEYKCKVSNKALPAPIEKTISKAKGQPREPQVYTLPPSRDELTKNQVSLTCLVKGFYPSDIAVEWESNGQPENNYKTTPPVLDSDGSFFLYSKLTVDKSRWQQGNVFSCSVMHEALHNHYTQKSLSLSPGK

SEQ ID NO: 7 - protein, 452 aa, synthetic construct
  CHAIN 1..452: note = cTF-hFc
SGTTNTVAAYNLTWKSTNFKTILEWEPKPINQVYTVQISTKSGDWKSKCFYTADTECDLTDEIVKDVKQTYLARVFSYPAGHVESTGSTEEPPYENSPEFTPYLETNLGQPTIQSFEQVGTKVNVTVQDEWTLVRRNDTFLSLRDVFGKDLIYTLYYWKSSSSGKKTAKTNTNEFLIDVDKGENYCFSVQAVIPSRRTANRKSTDSPVECMGHEKGESREEPKSSDKTHTCPPCPAPELLGGPSVFLFPPKPKDTLMISRTPEVTCVVVDVSHEDPEVKFNWYVDGVEVHNAKTKPREEQYNSTYRVVSVLTVLHQDWLNGKEYKCKVSNKALPAPIEKTISKAKGQPREPQVYTLPPSRDELTKNQVSLTCLVKGFYPSDIAVEWESNGQPENNYKTTPPVLDSDGSFFLYSKLTVDKSRWQQGNVFSCSVMHEALHNHYTQKSLSLSPGK

SEQ ID NO: 8 - protein, 228 aa, synthetic construct
  CHAIN 1..228: note = cTF-his
SGTTNTVAAYNLTWKSTNFKTILEWEPKPINQVYTVQISTKSGDWKSKCFYTADTECDLTDEIVKDVKQTYLARVFSYPAGHVESTGSTEEPPYENSPEFTPYLETNLGQPTIQSFEQVGTKVNVTVQDEWTLVRRNDTFLSLRDVFGKDLIYTLYYWKSSSSGKKTAKTNTNEFLIDVDKGENYCFSVQAVIPSRRTANRKSTDSPVECMGHEKGESRETGHHHHHH

SEQ ID NO: 9 - protein, 232 aa, synthetic construct
  CHAIN 1..232: note = Rat TF ECD-His
AGTPPGKAFNLTWISTDFKTILEWQPKPTNYTYTVQISDRSRNWKYKCTGTTDTECDLTDEIVKDVNWTYEARVLSVPWRNSTHGKETLFGTHGEEPPFTNARKFLPYRDTKIGQPVIQKYEQGGTKLKVTVKDSFTLVRKNGTFLTLRQVFGNDLGYILTYRKDSSTGRKTNTTHTNEFLIDVEKGVSYCFFAQAVIFSRKTNHKSPESITKCTEQWKSVLGETGHHHHHH

SEQ ID NO: 10 - protein, 231 aa, synthetic construct
  CHAIN 1..231: note = Mouse TF ECD-His
AGIPEKAFNLTWISTDFKTILEWQPKPTNYTYTVQISDRSRNWKNKCFSTTDTECDLTDEIVKDVTWAYEAKVLSVPRRNSVHGDGDQLVIHGEEPPFTNAPKFLPYRDTNLGQPVIQQFEQDGRKLNVVVKDSLTLVRKNGTFLTLRQVFGKDLGYIITYRKGSSTGKKTNITNTNEFSIDVEEGVSYCFFVQAMIFSRKTNQNSPGSSTVCTEQWKSFLGETGHHHHHH

SEQ ID NO: 11 - protein, 252 aa, synthetic construct
  CHAIN 1..252: note = HuRatTF
MAIPMRPRLLAALAPTFLGFLLLQVAVGAGTPPGKAFNLTWISADFKTILAWQPKPTNYTYTVQISTKSGDWKYKCTGTTDTECALTDEIVKDVKQTYLARVLSVPWRNSTHGKETLFGTHGEEPPFTNAPEFTPYLETNLGAPTIQSFEQVGTKVNVTVEDERTLVRRNNTFLSLRDVFGKDLIYTLAYWKSSSSGAKTAATNTNEFLIDVDKGENYCFSVQAVIPSRTVNRASTDSPVECMGQEHHHHHH

SEQ ID NO: 12 - protein, 566 aa, synthetic construct
  CHAIN 1..566: note = Human TF-2A-EGFP
METPAWPRVPRPETAVARTLLLGWVFAQVAGASGTTNTVAAYNLTWKSTNFKTILEWEPKPVNQVYTVQISTKSGDWKSKCFYTTDTECDLTDEIVKDVKQTYLARVFSYPAGNVESTGSAGEPLYENSPEFTPYLETNLGQPTIQSFEQVGTKVNVTVEDERTLVRRNNTFLSLRDVFGKDLIYTLYYWKSSSSGKKTAKTNTNEFLIDVDKGENYCFSVQAVIPSRTVNRKSTDSPVECMGQEKGEFREIFYIIGAVAFVVIILVIILAISLHKCRKAGVGQSWKENSPLNVSTSKIVAPVKQTLNFDLLKLAGDVESNPGPGSTMVSKGEELFTGVVPILVELDGDVNGHKFSVSGEGEGDATYGKLTLKFICTTGKLPVPWPTLVTTLTYGVQCFSRYPDHMKQHDFFKSAMPEGYVQERTIFFKDDGNYKTRAEVKFEGDTLVNRIELKGIDFKEDGNILGHKLEYNYNSHNVYIMADKQKNGIKVNFKIRHNIEDGSVQLADHYQQNTPIGDGPVLLPDNHYLSTQSALSKDPNEKRDHMVLLEFVTAAGITLGMDELYK

SEQ ID NO: 13 - protein, 567 aa, synthetic construct
  CHAIN 1..567: note = Cyno TF-2A-EGFP
METPAWPRVPRPETAVARTLLLGWVFAQVAGASGTTNTVAAYNLTWKSTNFKTILEWEPKPINQVYTVQISTKSGDWKSKCFYTADTECDLTDEIVKDVKQTYLARVFSYPAGHVESTGSTEEPPYENSPEFTPYLETNLGQPTIQSFEQVGTKVNVTVQDEWTLVRRNDTFLSLRDVFGKDLIYTLYYWKSSSSGKKTAKTNTNEFLIDVDKGENYCFSVQAVIPSRRTANRKSTDSPVECMGHEKGESREIFYIIGAVVFVVIILVIILAISLHKCKKARVGRSWKENSPLNVATSKIVAPVKQTLNFDLLKLAGDVESNPGPGSTMVSKGEELFTGVVPILVELDGDVNGHKFSVSGEGEGDATYGKLTLKFICTTGKLPVPWPTLVTTLTYGVQCFSRYPDHMKQHDFFKSAMPEGYVQERTIFFKDDGNYKTRAEVKFEGDTLVNRIELKGIDFKEDGNILGHKLEYNYNSHNVYIMADKQKNGIKVNFKIRHNIEDGSVQLADHYQQNTPIGDGPVLLPDNHYLSTQSALSKDPNEKRDHMVLLEFVTAAGITLGMDELYK

SEQ ID NO: 14 - protein, 41 aa, synthetic construct
  REGION 1..41: note = hTF1
METPAWPRVPRPETAVARTLLLGWVFAQVAGASGTTNTVAA

SEQ ID NO: 15 - protein, 43 aa, synthetic construct
  REGION 1..43: note = hTF2
YNLTWKSTNFKTILEWEPKPVNQVYTVQISTKSGDWKSKCFYT

SEQ ID NO: 16 - protein, 38 aa, synthetic construct
  REGION 1..38: note = hTF3
TDTECDLTDEIVKDVKQTYLARVFSYPAGNVESTGSAG

SEQ ID NO: 17 - protein, 15 aa, synthetic construct
  REGION 1..15: note = hTF4
EPLYENSPEFTPYLE

SEQ ID NO: 18 - protein, 47 aa, synthetic construct
  REGION 1..47: note = hTF7
TNLGQPTIQSFEQVGTKVNVTVEDERTLVRRNNTFLSLRDVFGKDLI

SEQ ID NO: 19 - protein, 41 aa, synthetic construct
  REGION 1..41: note = hTF5
YTLYYWKSSSSGKKTAKTNTNEFLIDVDKGENYCFSVQAVI

SEQ ID NO: 20 - protein, 25 aa, synthetic construct
  REGION 1..25: note = hTF6
PSRTVNRKSTDSPVECMGQEKGEFR

SEQ ID NO: 21 - protein, 560 aa, synthetic construct
  CHAIN 1..560: note = hTF1
MAILVRPRLLAALAPTFLGCLLLQVIAGAGIPEKAYNLTWKSTNFKTILEWEPKPVNQVYTVQISTKSGDWKSKCFYTTDTECDLTDEIVKDVKQTYLARVFSYPAGNVESTGSAGEPLYENSPEFTPYLETNLGQPTIQSFEQVGTKVNVTVEDERTLVRRNNTFLSLRDVFGKDLIYTLYYWKSSSSGKKTAKTNTNEFLIDVDKGENYCFSVQAVIPSRTVNRKSTDSPVECMGQEKGEFREIFYIIGAVAFVVIILVIILAISLHKCRKAGVGQSWKENSPLNVSTSKIVAPVKQTLNFDLLKLAGDVESNPGPGSTMVSKGEELFTGVVPILVELDGDVNGHKFSVSGEGEGDATYGKLTLKFICTTGKLPVPWPTLVTTLTYGVQCFSRYPDHMKQHDFFKSAMPEGYVQERTIFFKDDGNYKTRAEVKFEGDTLVNRIELKGIDFKEDGNILGHKLEYNYNSHNVYIMADKQKNGIKVNFKIRHNIEDGSVQLADHYQQNTPIGDGPVLLPDNHYLSTQSALSKDPNEKRDHMVLLEFVTAAGITLGMDELYK

SEQ ID NO: 22 - protein, 566 aa, synthetic construct
  CHAIN 1..566: note = hTF2
METPAWPRVPRPETAVARTLLLGWVFAQVAGASGTTNTVAAFNLTWISTDFKTILEWQPKPTNYTYTVQISDRSRNWKNKCFSTTDTECDLTDEIVKDVKQTYLARVFSYPAGNVESTGSAGEPLYENSPEFTPYLETNLGQPTIQSFEQVGTKVNVTVEDERTLVRRNNTFLSLRDVFGKDLIYTLYYWKSSSSGKKTAKTNTNEFLIDVDKGENYCFSVQAVIPSRTVNRKSTDSPVECMGQEKGEFREIFYIIGAVAFVVIILVIILAISLHKCRKAGVGQSWKENSPLNVSTSKIVAPVKQTLNFDLLKLAGDVESNPGPGSTMVSKGEELFTGVVPILVELDGDVNGHKFSVSGEGEGDATYGKLTLKFICTTGKLPVPWPTLVTTLTYGVQCFSRYPDHMKQHDFFKSAMPEGYVQERTIFFKDDGNYKTRAEVKFEGDTLVNRIELKGIDFKEDGNILGHKLEYNYNSHNVYIMADKQKNGIKVNFKIRHNIEDGSVQLADHYQQNTPIGDGPVLLPDNHYLSTQSALSKDPNEKRDHMVLLEFVTAAGITLGMDELYK

SEQ ID NO: 23 - protein, 572 aa, synthetic construct
  CHAIN 1..572: note = hTF3
METPAWPRVPRPETAVARTLLLGWVFAQVAGASGTTNTVAAYNLTWKSTNFKTILEWEPKPVNQVYTVQISTKSGDWKSKCFYTTDTECDLTDEIVKDVTWAYEAKVLSVPRRNSVHGDGDQLVIHGEEPLYENSPEFTPYLETNLGQPTIQSFEQVGTKVNVTVEDERTLVRRNNTFLSLRDVFGKDLIYTLYYWKSSSSGKKTAKTNTNEFLIDVDKGENYCFSVQAVIPSRTVNRKSTDSPVECMGQEKGEFREIFYIIGAVAFVVIILVIILAISLHKCRKAGVGQSWKENSPLNVSTSKIVAPVKQTLNFDLLKLAGDVESNPGPGSTMVSKGEELFTGVVPILVELDGDVNGHKFSVSGEGEGDATYGKLTLKFICTTGKLPVPWPTLVTTLTYGVQCFSRYPDHMKQHDFFKSAMPEGYVQERTIFFKDDGNYKTRAEVKFEGDTLVNRIELKGIDFKEDGNILGHKLEYNYNSHNVYIMADKQKNGIKVNFKIRHNIEDGSVQLADHYQQNTPIGDGPVLLPDNHYLSTQSALSKDPNEKRDHMVLLEFVTAAGITLGMDELYK

SEQ ID NO: 24 - protein, 566 aa, synthetic construct
  CHAIN 1..566: note = hTF4
METPAWPRVPRPETAVARTLLLGWVFAQVAGASGTTNTVAAYNLTWKSTNFKTILEWEPKPVNQVYTVQISTKSGDWKSKCFYTTDTECDLTDEIVKDVKQTYLARVFSYPAGNVESTGSAGEPPFTNAPKFLPYRDTNLGQPTIQSFEQVGTKVNVTVEDERTLVRRNNTFLSLRDVFGKDLIYTLYYWKSSSSGKKTAKTNTNEFLIDVDKGENYCFSVQAVIPSRTVNRKSTDSPVECMGQEKGEFREIFYIIGAVAFVVIILVIILAISLHKCRKAGVGQSWKENSPLNVSTSKIVAPVKQTLNFDLLKLAGDVESNPGPGSTMVSKGEELFTGVVPILVELDGDVNGHKFSVSGEGEGDATYGKLTLKFICTTGKLPVPWPTLVTTLTYGVQCFSRYPDHMKQHDFFKSAMPEGYVQERTIFFKDDGNYKTRAEVKFEGDTLVNRIELKGIDFKEDGNILGHKLEYNYNSHNVYIMADKQKNGIKVNFKIRHNIEDGSVQLADHYQQNTPIGDGPVLLPDNHYLSTQSALSKDPNEKRDHMVLLEFVTAAGITLGMDELYK

SEQ ID NO: 25 - protein, 566 aa, synthetic construct
  CHAIN 1..566: note = hTF7
METPAWPRVPRPETAVARTLLLGWVFAQVAGASGTTNTVAAYNLTWKSTNFKTILEWEPKPVNQVYTVQISTKSGDWKSKCFYTTDTECDLTDEIVKDVKQTYLARVFSYPAGNVESTGSAGEPLYENSPEFTPYLETNLGQPVIQQFEQDGRKLNVVVKDSLTLVRKNGTFLTLRQVFGKDLGYTLYYWKSSSSGKKTAKTNTNEFLIDVDKGENYCFSVQAVIPSRTVNRKSTDSPVECMGQEKGEFREIFYIIGAVAFVVIILVIILAISLHKCRKAGVGQSWKENSPLNVSTSKIVAPVKQTLNFDLLKLAGDVESNPGPGSTMVSKGEELFTGVVPILVELDGDVNGHKFSVSGEGEGDATYGKLTLKFICTTGKLPVPWPTLVTTLTYGVQCFSRYPDHMKQHDFFKSAMPEGYVQERTIFFKDDGNYKTRAEVKFEGDTLVNRIELKGIDFKEDGNILGHKLEYNYNSHNVYIMADKQKNGIKVNFKIRHNIEDGSVQLADHYQQNTPIGDGPVLLPDNHYLSTQSALSKDPNEKRDHMVLLEFVTAAGITLGMDELYK

SEQ ID NO: 26 - protein, 566 aa, synthetic construct
  CHAIN 1..566: note = hTF5
METPAWPRVPRPETAVARTLLLGWVFAQVAGASGTTNTVAAYNLTWKSTNFKTILEWEPKPVNQVYTVQISTKSGDWKSKCFYTTDTECDLTDEIVKDVKQTYLARVFSYPAGNVESTGSAGEPLYENSPEFTPYLETNLGQPTIQSFEQVGTKVNVTVEDERTLVRRNNTFLSLRDVFGKDLIYIITYRKGSSTGKKTNITNTNEFSIDVEEGVSYCFFVQAMIPSRTVNRKSTDSPVECMGQEKGEFREIFYIIGAVAFVVIILVIILAISLHKCRKAGVGQSWKENSPLNVSTSKIVAPVKQTLNFDLLKLAGDVESNPGPGSTMVSKGEELFTGVVPILVELDGDVNGHKFSVSGEGEGDATYGKLTLKFICTTGKLPVPWPTLVTTLTYGVQCFSRYPDHMKQHDFFKSAMPEGYVQERTIFFKDDGNYKTRAEVKFEGDTLVNRIELKGIDFKEDGNILGHKLEYNYNSHNVYIMADKQKNGIKVNFKIRHNIEDGSVQLADHYQQNTPIGDGPVLLPDNHYLSTQSALSKDPNEKRDHMVLLEFVTAAGITLGMDELYK

SEQ ID NO: 27 - protein, 566 aa, synthetic construct
  CHAIN 1..566: note = hTF6
METPAWPRVPRPETAVARTLLLGWVFAQVAGASGTTNTVAAYNLTWKSTNFKTILEWEPKPVNQVYTVQISTKSGDWKSKCFYTTDTECDLTDEIVKDVKQTYLARVFSYPAGNVESTGSAGEPLYENSPEFTPYLETNLGQPTIQSFEQVGTKVNVTVEDERTLVRRNNTFLSLRDVFGKDLIYTLYYWKSSSSGKKTAKTNTNEFLIDVDKGENYCFSVQAVIFSRKTNQNSPGSSTVCTEQWKSFLGEIFYIIGAVAFVVIILVIILAISLHKCRKAGVGQSWKENSPLNVSTSKIVAPVKQTLNFDLLKLAGDVESNPGPGSTMVSKGEELFTGVVPILVELDGDVNGHKFSVSGEGEGDATYGKLTLKFICTTGKLPVPWPTLVTTLTYGVQCFSRYPDHMKQHDFFKSAMPEGYVQERTIFFKDDGNYKTRAEVKFEGDTLVNRIELKGIDFKEDGNILGHKLEYNYNSHNVYIMADKQKNGIKVNFKIRHNIEDGSVQLADHYQQNTPIGDGPVLLPDNHYLSTQSALSKDPNEKRDHMVLLEFVTAAGITLGMDELYK

SEQ ID NO: 28 - protein, 448 aa, synthetic construct
  CHAIN 1..448: note = TF011-HC
EVQLLESGGGLVQPGGSLRLSCAASGFTFSNYAMSWVRQAPGKGLEWVSSISGSGDYTYYTDSVKGRFTISRDNSKNTLYLQMNSLRAEDTAVYYCARSPWGYYLDSWGQGTLVTVSSASTKGPSVFPLAPSSKSTSGGTAALGCLVKDYFPEPVTVSWNSGALTSGVHTFPAVLQSSGLYSLSSVVTVPSSSLGTQTYICNVNHKPSNTKVDKRVEPKSCDKTHTCPPCPAPELLGGPSVFLFPPKPKDTLMISRTPEVTCVVVDVSHEDPEVKFNWYVDGVEVHNAKTKPREEQYNSTYRVVSVLTVLHQDWLNGKEYKCKVSNKALPAPIEKTISKAKGQPREPQVYTLPPSREEMTKNQVSLTCLVKGFYPSDIAVEWESNGQPENNYKTTPPVLDSDGSFFLYSKLTVDKSRWQQGNVFSCSVMHEALHNHYTQKSLSLSPGK

SEQ ID NO: 29 - protein, 214 aa, synthetic construct
  CHAIN 1..214: note = TF011-LC
DIQMTQSPPSLSASAGDRVTITCRASQGISSRLAWYQQKPEKAPKSLIYAASSLQSGVPSRFSGSGSGTDFTLTISSLQPEDFATYYCQQYNSYPYTFGQGTKLEIKRTVAAPSVFIFPPSDEQLKSGTASVVCLLNNFYPREAKVQWKVDNALQSGNSQESVTEQDSKDSTYSLSSTLTLSKADYEKHKVYACEVTHQGLSSPVTKSFNRGEC

SEQ ID NO: 30 - protein, 447 aa, synthetic construct
  CHAIN 1..447: note = H39-HC
EVQLVQSGAEVKKPGESLKISCKGSGYSFTSYWMNWVRQMPGKGLEWMGMIYPADSETRLNQKFKDQATLSVDKSISTAYLQWSSLKASDTAMYYCAREDYGSSDYWGQGTTVTVSSASTKGPSVFPLAPSSKSTSGGTAALGCLVKDYFPEPVTVSWNSGALTSGVHTFPAVLQSSGLYSLSSVVTVPSSSLGTQTYICNVNHKPSNTKVDKKVEPKSCDKTHTCPPCPAPELLGGPSVFLFPPKPKDTLMISRTPEVTCVVVDVSHEDPEVKFNWYVDGVEVHNAKTKPREEQYNSTYRVVSVLTVLHQDWLNGKEYKCKVSNKALPAPIEKTISKAKGQPREPQVYTLPPSRDELTKNQVSLTCLVKGFYPSDIAVEWESNGQPENNYKTTPPVLDSDGSFFLYSKLTVDKSRWQQGNVFSCSVMHEALHNHYTQKSLSLSPGK

SEQ ID NO: 31 - protein, 213 aa, synthetic construct
  CHAIN 1..213: note = H39-LC
DIQLTQSPSSLSASVGDRVTITCSASSSVSYMNWYQQKPGKSPKIWIYGISNLASGVPSRFSGSGSGTDFTLTISSLQPEDFATYYCQQKSSFPWTFGGGTKVEIKRTVAAPSVFIFPPSDEQLKSGTASVVCLLNNFYPREAKVQWKVDNALQSGNSQESVTEQDSKDSTYSLSSTLTLSKADYEKHKVYACEVTHQGLSSPVTKSFNRGEC

SEQ ID NO: 32 - protein, 450 aa, synthetic construct
  CHAIN 1..450: note = 10H10-HC
QVHLQQSGAELMKPGASVKISCKASGYTFITYWIEWVKQRPGHGLEWIGDILPGSGSTNYNENFKGKATFTADSSSNTAYMQLSSLTSEDSAVYYCARSGYYGNSGFAYWGQGTLVTVSAASTKGPSVFPLAPSSKSTSGGTAALGCLVKDYFPEPVTVSWNSGALTSGVHTFPAVLQSSGLYSLSSVVTVPSSSLGTQTYICNVNHKPSNTKVDKKVEPKSCDKTHTCPPCPAPELLGGPSVFLFPPKPKDTLMISRTPEVTCVVVDVSHEDPEVKFNWYVDGVEVHNAKTKPREEQYNSTYRVVSVLTVLHQDWLNGKEYKCKVSNKALPAPIEKTISKAKGQPREPQVYTLPPSRDELTKNQVSLTCLVKGFYPSDIAVEWESNGQPENNYKTTPPVLDSDGSFFLYSKLTVDKSRWQQGNVFSCSVMHEALHNHYTQKSLSLSPGK

SEQ ID NO: 33 - protein, 220 aa, synthetic construct
  CHAIN 1..220: note = 10H10-LC
DIVMTQSPSSLTVTAGEKVTMSCKSSQSLLSSGNQKNYLTWYQQIPGQPPKLLIYWASTRESGVPDRFTGSGSGTDFTLTINSVQAEDLAVYYCQNDYTYPLTFGAGTKLELKRTVAAPSVFIFPPSDEQLKSGTASVVCLLNNFYPREAKVQWKVDNALQSGNSQESVTEQDSKDSTYSLSSTLTLSKADYEKHKVYACEVTHQGLSSPVTKSFNRGEC

SEQ ID NO: 34 - protein, 448 aa, synthetic construct
  CHAIN 1..448: note = TF011-mIgG2a-HC
EVQLLESGGGLVQPGGSLRLSCAASGFTFSNYAMSWVRQAPGKGLEWVSSISGSGDYTYYTDSVKGRFTISRDNSKNTLYLQMNSLRAEDTAVYYCARSPWGYYLDSWGQGTLVTVSSAKTTAPSVYPLAPVCGDTTGSSVTLGCLVKGYFPEPVTLTWNSGSLSSGVHTFPAVLQSDLYTLSSSVTVTSSTWPSQSITCNVAHPASSTKVDKKIEPRGPTIKPCPPCKCPAPNLLGGPSVFIFPPKIKDVLMISLSPIVTCVVVDVSEDDPDVQISWFVNNVEVHTAQTQTHREDYNSTLRVVSALPIQHQDWMSGKEFKCKVNNKDLPAPIERTISKPKGSVRAPQVYVLPPPEEEMTKKQVTLTCMVTDFMPEDIYVEWTNNGKTELNYKNTEPVLDSDGSYFMYSKLRVEKKNWVERNSYSCSVVHEGLHNHHTTKSFSRTPGK

SEQ ID NO: 35 - protein, 214 aa, synthetic construct
  CHAIN 1..214: note = TF011-mkappa
DIQMTQSPPSLSASAGDRVTITCRASQGISSRLAWYQQKPEKAPKSLIYAASSLQSGVPSRFSGSGSGTDFTLTISSLQPEDFATYYCQQYNSYPYTFGQGTKLEIKRADAAPTVSIFPPSSEQLTSGGASVVCFLNNFYPKDINVKWKIDGSERQNGVLNSWTDQDSKDSTYSMSSTLTLTKDEYERHNSYTCEATHKTSTSPIVKSFNRNEC

SEQ ID NO: 36 - protein, 120 aa, Mus musculus
  REGION 1..120: note = 67#-VH
QVQLKQSGPGLVQPSQSLSITCIVSGFSLTNYGVNWVRQSPRKGLEWLGVIWSRGNTDYNAAFISRLIISKDNSKSQVFLKMNRLQADDTAIYYCARKDAVVATDALDYWGQGTSVTVSS

SEQ ID NO: 37 - protein, 107 aa, Mus musculus
  CHAIN 1..107: note = 67#-VL
DIVMTQSHKFMSTSLGDRVSITCKASQDVSTAVAWYQQKPGQSPKLLIYSTSYRYTGVPDRFTGSGSGTDFTFTISSVQAEDLAVYYCQQHYSTPYTFGGGTKLEIK

SEQ ID NO: 38 - protein, 118 aa, Mus musculus
  REGION 1..118: note = 310#-VH
EVQLQQSGPELVKPGASLKISCKASGYSFTGYYMNWVKQSPEKSLEWIGEINPSTGGSTYNQKFKAKATLTVDQSSNTAYMQLKSLTSEDSAVYYCARRELGGPFGYWGQGTPVTVSA

SEQ ID NO: 39 - protein, 107 aa, Mus musculus
  REGION 1..107: note = 310#-VL
SIVMTQTPKFLLVSSGDRVTITCKASQSVSNGIAWYQQKPGQSPKLLIYFASNRYTGVPDRFTGSGYGTDFTFTISTVQAEDLAVYFCQQDYSSPWTFGGGTKLEIK

SEQ ID NO: 40 - protein, 5 aa, Mus musculus
  REGION 1..5: note = 67-HCDR1
NYGVN

SEQ ID NO: 41 - protein, 16 aa, Mus musculus
  REGION 1..16: note = 67-HCDR2
VIWSRGNTDYNAAFIS

SEQ ID NO: 42 - protein, 12 aa, Mus musculus
  REGION 1..12: note = 67-HCDR3
KDAVVATDALDY

SEQ ID NO: 43 - protein, 11 aa, Mus musculus
  REGION 1..11: note = 67-LCDR1
KASQDVSTAVA

SEQ ID NO: 44 - protein, 7 aa, Mus musculus
  REGION 1..7: note = 67-LCDR2
STSYRYT

SEQ ID NO: 45 - protein, 9 aa, Mus musculus
  REGION 1..9: note = 67-HCDR3
QQHYSTPYT

SEQ ID NO: 46 - protein, 5 aa, Mus musculus
  REGION 1..5: note = 310-HCDR1
GYYMN

SEQ ID NO: 47 - protein, 17 aa, Mus musculus
  REGION 1..17: note = 310-HCDR2
EINPSTGGSTYNQKFKA

SEQ ID NO: 48 - protein, 9 aa, Mus musculus
  REGION 1..9: note = 310-HCDR3
RELGGPFGY

SEQ ID NO: 49 - protein, 11 aa, Mus musculus
  REGION 1..11: note = 310-LCDR1
KASQSVSNGIA

SEQ ID NO: 50 - protein, 7 aa, Mus musculus
  REGION 1..7: note = 310-LCDR2
FASNRYT

SEQ ID NO: 51 - protein, 9 aa, Mus musculus
  REGION 1..9: note = 310-LCDR3
QQDYSSPWT

SEQ ID NO: 52 - protein, 118 aa, synthetic construct
  REGION 1..118: note = hu310-VH1
EVQLVQSGAEVKKPGASVKVSCKASGYSFTGYYMNWVRQAPGQGLEWMGEINPSTGGSTYNQKFKARVTMTVDQSTSTVYMELSSLRSEDTAVYYCARRELGGPFGYWGQGTTVTVSS

SEQ ID NO: 53 - protein, 107 aa, synthetic construct
  REGION 1..107: note = hu310-VL2
SIVMTQSPDSLAVSLGERATINCKASQSVSNGIAWYQQKPGQSPKLLIYFASNRYTGVPDRFSGSGYGTDFTLTISSLQAEDVAVYYCQQDYSSPWTFGGGTKVEIK

SEQ ID NO: 54 - protein, 330 aa, Homo sapiens [sequence omitted]

SEQ ID NO: 55 - protein, 107 aa, Homo sapiens [sequence omitted]

SEQ ID NO: 56 - protein, 448 aa, synthetic construct
  CHAIN 1..448: note = hu310-1/hu310-2/hu310-3/hu310-4/hu310-5/hu310-6/hu310-7/hu310-8-HC
EVQLVQSGAEVKKPGASVKVSCKASGYSFTGYYMNWVRQAPGQGLEWMGEINPSTGGSTYNQKFKARVTMTVDQSTSTVYMELSSLRSEDTAVYYCARRELGGPFGYWGQGTTVTVSSASTKGPSVFPLAPSSKSTSGGTAALGCLVKDYFPEPVTVSWNSGALTSGVHTFPAVLQSSGLYSLSSVVTVPSSSLGTQTYICNVNHKPSNTKVDKKVEPKSCDKTHTCPPCPAPELLGGPSVFLFPPKPKDTLMISRTPEVTCVVVDVSHEDPEVKFNWYVDGVEVHNAKTKPREEQYNSTYRVVSVLTVLHQDWLNGKEYKCKVSNKALPAPIEKTISKAKGQPREPQVYTLPPSRDELTKNQVSLTCLVKGFYPSDIAVEWESNGQPENNYKTTPPVLDSDGSFFLYSKLTVDKSRWQQGNVFSCSVMHEALHNHYTQKSLSLSPGK

SEQ ID NO: 57 - protein, 214 aa, synthetic construct
  CHAIN 1..214: note = hu310-2/hu310-10-LC
SIVMTQSPDSLAVSLGERATINCKASQSVSNGIAWYQQKPGQSPKLLIYFASNRYTGVPDRFSGSGYGTDFTLTISSLQAEDVAVYYCQQDYSSPWTFGGGTKVEIKRTVAAPSVFIFPPSDEQLKSGTASVVCLLNNFYPREAKVQWKVDNALQSGNSQESVTEQDSKDSTYSLSSTLTLSKADYEKHKVYACEVTHQGLSSPVTKSFNRGEC

SEQ ID NO: 58 - protein, 120 aa, synthetic construct
  REGION 1..120: note = hu67-VH3
EVQLQESGPGLVKPSQTLSLTCTVSGFSLTNYGVNWIRQPPGKGLEWIGVIWSRGNTDYNAAFISRVTISKDTSKNQVSLKLSSVTAADTAVYYCARKDAVVATDALDYWGQGTTVTVSS

SEQ ID NO: 59 - protein, 107 aa, synthetic construct
  REGION 1..107: note = 67VL-VL3
DIQMTQSPSSLSASVGDRVTITCKASQDVSTAVAWYQQKPGKAPKLLIYSTSYRYTGVPSRFSGSGSGTDFTFTISSLQPEDIATYYCQQHYSTPYTFGGGTKVEIK

SEQ ID NO: 60 - protein, 450 aa, synthetic construct
  CHAIN 1..450: note = hu67-3/hu67-7/hu67-11/hu67-15-HC
EVQLQESGPGLVKPSQTLSLTCTVSGFSLTNYGVNWIRQPPGKGLEWIGVIWSRGNTDYNAAFISRVTISKDTSKNQVSLKLSSVTAADTAVYYCARKDAVVATDALDYWGQGTTVTVSSASTKGPSVFPLAPSSKSTSGGTAALGCLVKDYFPEPVTVSWNSGALTSGVHTFPAVLQSSGLYSLSSVVTVPSSSLGTQTYICNVNHKPSNTKVDKKVEPKSCDKTHTCPPCPAPELLGGPSVFLFPPKPKDTLMISRTPEVTCVVVDVSHEDPEVKFNWYVDGVEVHNAKTKPREEQYNSTYRVVSVLTVLHQDWLNGKEYKCKVSNKALPAPIEKTISKAKGQPREPQVYTLPPSRDELTKNQVSLTCLVKGFYPSDIAVEWESNGQPENNYKTTPPVLDSDGSFFLYSKLTVDKSRWQQGNVFSCSVMHEALHNHYTQKSLSLSPGK

SEQ ID NO: 61 - protein, 214 aa, synthetic construct
  CHAIN 1..214: note = hu67-9/hu67-10/hu67-11/hu67-12-LC
DIQMTQSPSSLSASVGDRVTITCKASQDVSTAVAWYQQKPGKAPKLLIYSTSYRYTGVPSRFSGSGSGTDFTFTISSLQPEDIATYYCQQHYSTPYTFGGGTKVEIKRTVAAPSVFIFPPSDEQLKSGTASVVCLLNNFYPREAKVQWKVDNALQSGNSQESVTEQDSKDSTYSLSSTLTLSKADYEKHKVYACEVTHQGLSSPVTKSFNRGEC

SEQ ID NO: 62 - protein, 120 aa, synthetic construct
  REGION 1..120: note = hu67Y116/ hu67Y118-VH
EVQLQESGPGLVKPSQTLSLTCTVSGFSLTNYGVNWIRQSPGKGLEWIGVIWSRGNTDYNAAFKSRVTISKDTSKNQVSLKLSSVTAADTAVYYCARKDAIVATDALDYWGQGTTVTVSS

SEQ ID NO: 63 - protein, 107 aa, synthetic construct
  REGION 1..107: note = hu67Y116-VL
DIQMTQSPSSLSASVGDRVTITCKASQDVQTAVAWYQQKPGKAPKLLIYSTHYRYTGVPSRFSGSGSGTDFTFTISSLQPEDIATYYCLQSYTLPFSFGGGTKVEIK

SEQ ID NO: 64 - protein, 16 aa, synthetic construct
  REGION 1..16: note = hu67Y116-HCDR2
VIWSRGNTDYNAAFKS

SEQ ID NO: 65 - protein, 12 aa, synthetic construct
  REGION 1..12: note = hu67Y116-HCDR3
KDAIVATDALDY

SEQ ID NO: 66 - protein, 11 aa, synthetic construct
  REGION 1..11: note = hu67Y116-LCDR1
KASQDVQTAVA

SEQ ID NO: 67 - protein, 7 aa, synthetic construct
  REGION 1..7: note = hu67Y116-LCDR2
STHYRYT

SEQ ID NO: 68 - protein, 9 aa, synthetic construct
  REGION 1..9: note = hu67Y116-LCDR3
LQSYTLPFS

SEQ ID NO: 69 - protein, 450 aa, synthetic construct
  CHAIN 1..450: note = hu67Y116/ hu67Y118-HC
EVQLQESGPGLVKPSQTLSLTCTVSGFSLTNYGVNWIRQSPGKGLEWIGVIWSRGNTDYNAAFKSRVTISKDTSKNQVSLKLSSVTAADTAVYYCARKDAIVATDALDYWGQGTTVTVSSASTKGPSVFPLAPSSKSTSGGTAALGCLVKDYFPEPVTVSWNSGALTSGVHTFPAVLQSSGLYSLSSVVTVPSSSLGTQTYICNVNHKPSNTKVDKKVEPKSCDKTHTCPPCPAPELLGGPSVFLFPPKPKDTLMISRTPEVTCVVVDVSHEDPEVKFNWYVDGVEVHNAKTKPREEQYNSTYRVVSVLTVLHQDWLNGKEYKCKVSNKALPAPIEKTISKAKGQPREPQVYTLPPSRDELTKNQVSLTCLVKGFYPSDIAVEWESNGQPENNYKTTPPVLDSDGSFFLYSKLTVDKSRWQQGNVFSCSVMHEALHNHYTQKSLSLSPGK

SEQ ID NO: 70 - protein, 214 aa, synthetic construct
  CHAIN 1..214: note = hu67Y116-LC
DIQMTQSPSSLSASVGDRVTITCKASQDVQTAVAWYQQKPGKAPKLLIYSTHYRYTGVPSRFSGSGSGTDFTFTISSLQPEDIATYYCLQSYTLPFSFGGGTKVEIKRTVAAPSVFIFPPSDEQLKSGTASVVCLLNNFYPREAKVQWKVDNALQSGNSQESVTEQDSKDSTYSLSSTLTLSKADYEKHKVYACEVTHQGLSSPVTKSFNRGEC

SEQ ID NO: 71 - protein, 120 aa, synthetic construct
  REGION 1..120: note = hu10H10 VH11
EVQLVQSGSELKKPGASVKVSCKASGYTFITYWIEWVKQRPGQGLEWMGDILPYSGSTNYNENFKGRATFSADTSVSTAYLQISSLKAEDTAVYYCARSGYYGNSGFAYWGQGTLVTVSS

SEQ ID NO: 72 - protein, 113 aa, synthetic construct
  REGION 1..113: note = hu10H10 VL9
DIQMTQSPSSLSASVGDRVTITCQSSQSLLSSGNQKNYLTWYQQKPGKAPKLLIYWASTRESGVPSRFSGSGSGTDFTLTISSLQPEDFATYYCQNDYTYPLTFGQGTKLEIK

SEQ ID NO: 73 - protein, 5 aa, synthetic construct
  REGION 1..5: note = hu10H10-77-HCDR1
TYWIE

SEQ ID NO: 74 - protein, 17 aa, synthetic construct
  REGION 1..17: note = hu10H10-77-HCDR2
DILPYSGSTNYNENFKG

SEQ ID NO: 75 - protein, 11 aa, synthetic construct
  REGION 1..11: note = hu10H10-77-HCDR3
SGYYGNSGFAY

SEQ ID NO: 76 - protein, 17 aa, synthetic construct
  REGION 1..17: note = hu10H10-77-LCDR1
QSSQSLLSSGNQKNYLT

SEQ ID NO: 77 - protein, 7 aa, synthetic construct
  REGION 1..7: note = hu10H10-77-LCDR2
WASTRES

SEQ ID NO: 78 - protein, 9 aa, synthetic construct
  REGION 1..9: note = hu10H10-77-LCDR3
QNDYTYPLT

SEQ ID NO: 79 - protein, 450 aa, synthetic construct
  CHAIN 1..450: note = hu10H10-29/hu10H10-37/hu10H10-45//hu10H10-53/hu10H10-77-HC
EVQLVQSGSELKKPGASVKVSCKASGYTFITYWIEWVKQRPGQGLEWMGDILPYSGSTNYNENFKGRATFSADTSVSTAYLQISSLKAEDTAVYYCARSGYYGNSGFAYWGQGTLVTVSSASTKGPSVFPLAPSSKSTSGGTAALGCLVKDYFPEPVTVSWNSGALTSGVHTFPAVLQSSGLYSLSSVVTVPSSSLGTQTYICNVNHKPSNTKVDKKVEPKSCDKTHTCPPCPAPELLGGPSVFLFPPKPKDTLMISRTPEVTCVVVDVSHEDPEVKFNWYVDGVEVHNAKTKPREEQYNSTYRVVSVLTVLHQDWLNGKEYKCKVSNKALPAPIEKTISKAKGQPREPQVYTLPPSRDELTKNQVSLTCLVKGFYPSDIAVEWESNGQPENNYKTTPPVLDSDGSFFLYSKLTVDKSRWQQGNVFSCSVMHEALHNHYTQKSLSLSPGK

SEQ ID NO: 80 - protein, 220 aa, synthetic construct
  CHAIN 1..220: note = hu10H10-77-LC
DIQMTQSPSSLSASVGDRVTITCQSSQSLLSSGNQKNYLTWYQQKPGKAPKLLIYWASTRESGVPSRFSGSGSGTDFTLTISSLQPEDFATYYCQNDYTYPLTFGQGTKLEIKRTVAAPSVFIFPPSDEQLKSGTASVVCLLNNFYPREAKVQWKVDNALQSGNSQESVTEQDSKDSTYSLSSTLTLSKADYEKHKVYACEVTHQGLSSPVTKSFNRGEC

SEQ ID NO: 81 - protein, 107 aa, synthetic construct
  REGION 1..107: note = hu67Y118-VL
DIQMTQSPSSLSASVGDRVTITCKASQDVQTAVAWYQQKPGKAPKLLIYSTHYRYTGVPSRFSGSGSGTDFTFTISSLQPEDIATYYCLQLIGVPHTFGGGTKVEIK

SEQ ID NO: 82 - protein, 214 aa, synthetic construct
  CHAIN 1..214: note = hu67Y118-LC
DIQMTQSPSSLSASVGDRVTITCKASQDVQTAVAWYQQKPGKAPKLLIYSTHYRYTGVPSRFSGSGSGTDFTFTISSLQPEDIATYYCLQLIGVPHTFGGGTKVEIKRTVAAPSVFIFPPSDEQLKSGTASVVCLLNNFYPREAKVQWKVDNALQSGNSQESVTEQDSKDSTYSLSSTLTLSKADYEKHKVYACEVTHQGLSSPVTKSFNRGEC

SEQ ID NO: 83 - protein, 9 aa, synthetic construct
  REGION 1..9: note = hu67Y118-LCDR3
LQLIGVPHT

SEQ ID NO: 84 - protein, 120 aa, synthetic construct
  REGION 1..120: note = hu10H10 VH1
EVQLVQSGAEVKKPGASVKVSCKASGYTFITYWIEWVRQRPGQGLEWMGDILPGSGSTNYNENFKGRVTFTADTSTSTVYMQLSSLRSEDTAVYYCARSGYYGNSGFAYWGQGTLVTVSS

SEQ ID NO: 85 - protein, 120 aa, synthetic construct
  REGION 1..120: note = hu10H10 VH2
EVQLVQSGSELKKPGASVKVSCKASGYTFITYWIEWVRQRPGQGLEWMGDILPGSGSTNYNENFKGRAVFSADTSVSTAYLQISSLKAEDTAVYYCARSGYYGNSGFAYWGQGTLVTVSS

SEQ ID NO: 86 - protein, 120 aa, synthetic construct
  REGION 1..120: note = hu10H10 VH3
EVQLVQSGAEVKKPGASVKVSCKASIYTFITYWIEWVRQRPGQGLEWMGDILPGSGSTNYNENFKGRVTFTADTSTSTVYMQLSSLRSEDTAVYYCARSGYYGNSGFAYWGQGTLVTVSS

SEQ ID NO: 87 - protein, 120 aa, synthetic construct
  REGION 1..120: note = hu10H10 VH4
EVQLVQSGSELKKPGASVKVSCKASGFTFITYWIEWVRQRPGQGLEWMGDILPGSGSTNYNENFKGRAVFSADTSVSTAYLQISSLKAEDTAVYYCARSGYYGNSGFAYWGQGTLVTVSS

SEQ ID NO: 88 - protein, 120 aa, synthetic construct
  REGION 1..120: note = hu10H10 VH5
EVQLVQSGAEVKKPGASVKVSCKASGYTFITYWIEWVRQRPGQGLEWMGDILPGSGSSNYNENFKGRVTFTADTSTSTVYMQLSSLRSEDTAVYYCARSGYYGNSGFAYWGQGTLVTVSS

SEQ ID NO: 89 - protein, 120 aa, synthetic construct
  REGION 1..120: note = hu10H10 VH6
EVQLVQSGSELKKPGASVKVSCKASGYTFITYWIEWVRQRPGQGLEWMGDILPGSGSTNYNENFKGRAVFSADTSVSTAYLQISSLKAEDTAVYYCARSGYYGNSGFVYWGQGTLVTVSS

SEQ ID NO: 90 - protein, 120 aa, synthetic construct
  REGION 1..120: note = hu10H10 VH7
EVQLVQSGSELKKPGASVKVSCKASGYTFITYWIEWVKQRPGQGLEWMGDILPGSGSTNYNENFKGRATFSADTSVSTAYLQISSLKAEDTAVYYCARSGYYGNSGFAYWGQGTLVTVSS

SEQ ID NO: 91 - protein, 120 aa, synthetic construct
  REGION 1..120: note = hu10H10 VH8
EVQLVQSGSELKKPGASVKVSCKASGRTFITYWIEWVRQRPGQGLEWMGDILPGSGSTNYNENFKGRATFSADTSVSTAYLQISSLKAEDTAVYYCARSGYYGNSGFAYWGQGTLVTVSS

SEQ ID NO: 92 - protein, 120 aa, synthetic construct
  REGION 1..120: note = hu10H10 VH9
EVQLVQSGSELKKPGASVKVSCKASGYTFRTYWIEWVKQRPGQGLEWMGDILPGSGSTNYNENFKGRATFSADTSVSTAYLQISSLKAEDTAVYYCARSGYYGNSGFAYWGQGTLVTVSS

SEQ ID NO: 93 - protein, 120 aa, synthetic construct
  REGION 1..120: note = hu10H10 VH10
EVQLVQSGSELKKPGASVKVSCKASGYTFIEYWIEWVKQRPGQGLEWMGDILPGSGSTNYNENFKGRATFSADTSVSTAYLQISSLKAEDTAVYYCARSGYYGNSGFAYWGQGTLVTVSS

SEQ ID NO: 94 - protein, 120 aa, synthetic construct
  REGION 1..120: note = hu10H10 VH12
EVQLVQSGSELKKPGASVKVSCKASGYTFITYWIEWVKQRPGQGLEWMGDILPGHGSTNYNENFKGRATFSADTSVSTAYLQISSLKAEDTAVYYCARSGYYGNSGFAYWGQGTLVTVSS

SEQ ID NO: 95 - protein, 120 aa, synthetic construct
  REGION 1..120: note = hu10H10 VH13
EVQLVQSGSELKKPGASVKVSCKASGYTFITYWIEWVKQRPGQGLEWMGDILPGSGWTNYNENFKGRATFSADTSVSTAYLQISSLKAEDTAVYYCARSGYYGNSGFAYWGQGTLVTVSS

SEQ ID NO: 96 - protein, 120 aa, synthetic construct
  REGION 1..120: note = hu10H10 VH14
EVQLVQSGSELKKPGASVKVSCKASGYTFITYWIEWVRQRPGQGLEWMGDILPGSGWTNYNENFKGRAVFSADTSVSTAYLQISSLKAEDTAVYYCARSGYYGNSGFAYWGQGTLVTVSS

SEQ ID NO: 97 - protein, 113 aa, synthetic construct
  REGION 1..107: note = hu10H10 VL1
DIQMTQSPSSLSASVGDRVTITCKSSQSLLSSGNQKNYLTWYQQKPGKAPKLLIYWASTRESGVPSRFSGSGSGTDFTLTISSLQPEDFATYYCQNDYTYPLTFGQGTKLEIK

SEQ ID NO: 98 - protein, 113 aa, synthetic construct
  REGION 1..107: note = hu10H10 VL2
DIQMTQSPSSLSASVGDRVTITCRASQSILSSGNQKNYLTWYQQKPGKAPKLLIYWASTRESGVPSRFSGSGSGTDFTLTISSLQPEDFATYYCQNDYTYPLTFGQGTKLEIK

SEQ ID NO: 99 - protein, 113 aa, synthetic construct
  REGION 1..107: note = hu10H10 VL3
DIQMTQSPSSLSASVGDRVTITCKSSQSLLSSGNQKNYLTWYQQKPGKAPKLLIYWASTREEGVPSRFSGSGSGTDFTLTISSLQPEDFATYYCQNDYTYPLTFGQGTKLEIK

SEQ ID NO: 100 - protein, 113 aa, synthetic construct
  REGION 1..107: note = hu10H10 VL4
DIQMTQSPSSLSASVGDRVTITCKSSQSLLSSGNQKNYLTWYQQKPGKAPKLLIYWASTRESGVPSRFSGSGSGTDFTLTISSLQPEDFATYYCQNDYTYPLSFGQGTKLEIK

SEQ ID NO: 101 - protein, 113 aa, synthetic construct
  REGION 1..107: note = hu10H10 VL5
DIQMTQSPSSLSASVGDRVTITCKSSQSLLDSGNQKNYLTWYQQKPGKAPKLLIYWASTREEGVPSRFSGSGSGTDFTLTISSLQPEDFATYYCQNDYTYPLTFGQGTKLEIK

SEQ ID NO: 102 - protein, 113 aa, synthetic construct
  REGION 1..107: note = hu10H10 VL6
DIQMTQSPSSLSASVGDRVTITCKSSQSLLSSSNQKNYLTWYQQKPGKAPKLLIYWASTREEGVPSRFSGSGSGTDFTLTISSLQPEDFATYYCQNDYTYPLTFGQGTKLEIK

SEQ ID NO: 103 - protein, 448 aa, synthetic construct
  CHAIN 1..448: note = hIgG1-C25-HC
QVQLVQSGAEVKKPGASVKVSCKASGYTFTNSWIGWFRQAPGQGLEWIGDIYPGGGYTNYNEIFKGKATMTADTSTNTAYMELSSLRSEDTAVYYCSRGIPGYAMDYWGQGTLVTVSSASTKGPSVFPLAPSSKSTSGGTAALGCLVKDYFPEPVTVSWNSGALTSGVHTFPAVLQSSGLYSLSSVVTVPSSSLGTQTYICNVNHKPSNTKVDKKVEPKSCDKTHTCPPCPAPELLGGPSVFLFPPKPKDTLMISRTPEVTCVVVDVSHEDPEVKFNWYVDGVEVHNAKTKPREEQYNSTYRVVSVLTVLHQDWLNGKEYKCKVSNKALPAPIEKTISKAKGQPREPQVYTLPPSRDELTKNQVSLTCLVKGFYPSDIAVEWESNGQPENNYKTTPPVLDSDGSFFLYSKLTVDKSRWQQGNVFSCSVMHEALHNHYTQKSLSLSPGK

SEQ ID NO: 104 - protein, 220 aa, synthetic construct
  CHAIN 1..220: note = hIgG1-C25-LC
DIQMTQSPSSLSASVGDRVTMSCKSSQSLLNSGDQKNYLTWYQQKPGKAPKLLIYWASTGESGVPSRFSGSGSGTDFTFTISSLQPEDIATYYCQNDYSYPWTFGQGTKVEIKRTVAAPSVFIFPPSDEQLKSGTASVVCLLNNFYPREAKVQWKVDNALQSGNSQESVTEQDSKDSTYSLSSTLTLSKADYEKHKVYACEVTHQGLSSPVTKSFNRGEC

SEQ ID NO: 105 - protein, 4 aa, synthetic construct
  REGION 1..4: note = L3
GGFG

SEQ ID NO: 106 - protein, 453 aa, synthetic construct
  CHAIN 1..453: note = cTF-mFc
SGTTNTVAAYNLTWKSTNFKTILEWEPKPINQVYTVQISTKSGDWKSKCFYTADTECDLTDEIVKDVKQTYLARVFSYPAGHVESTGSTEEPPYENSPEFTPYLETNLGQPTIQSFEQVGTKVNVTVQDEWTLVRRNDTFLSLRDVFGKDLIYTLYYWKSSSSGKKTAKTNTNEFLIDVDKGENYCFSVQAVIPSRRTANRKSTDSPVECMGHEKGESREEPRGPTIKPCPPCKCPAPNLLGGPSVFIFPPKIKDVLMISLSPIVTCVVVDVSEDDPDVQISWFVNNVEVHTAQTQTHREDYNSTLRVVSALPIQHQDWMSGKEFKCKVNNKDLPAPIERTISKPKGSVRAPQVYVLPPPEEEMTKKQVTLTCMVTDFMPEDIYVEWTNNGKTELNYKNTEPVLDSDGSYFMYSKLRVEKKNWVERNSYSCSVVHEGLHNHHTTKSFSRTPGK

SEQ ID NO: 107 - protein, 450 aa, synthetic construct
  CHAIN 1..450: note = CH67-HC
QVQLKQSGPGLVQPSQSLSITCIVSGFSLTNYGVNWVRQSPRKGLEWLGVIWSRGNTDYNAAFISRLIISKDNSKSQVFLKMNRLQADDTAIYYCARKDAVVATDALDYWGQGTSVTVSSASTKGPSVFPLAPSSKSTSGGTAALGCLVKDYFPEPVTVSWNSGALTSGVHTFPAVLQSSGLYSLSSVVTVPSSSLGTQTYICNVNHKPSNTKVDKKVEPKSCDKTHTCPPCPAPELLGGPSVFLFPPKPKDTLMISRTPEVTCVVVDVSHEDPEVKFNWYVDGVEVHNAKTKPREEQYNSTYRVVSVLTVLHQDWLNGKEYKCKVSNKALPAPIEKTISKAKGQPREPQVYTLPPSRDELTKNQVSLTCLVKGFYPSDIAVEWESNGQPENNYKTTPPVLDSDGSFFLYSKLTVDKSRWQQGNVFSCSVMHEALHNHYTQKSLSLSPGK

SEQ ID NO: 108 - protein, 214 aa, synthetic construct
  CHAIN 1..214: note = CH67-LC
DIVMTQSHKFMSTSLGDRVSITCKASQDVSTAVAWYQQKPGQSPKLLIYSTSYRYTGVPDRFTGSGSGTDFTFTISSVQAEDLAVYYCQQHYSTPYTFGGGTKLEIKRTVAAPSVFIFPPSDEQLKSGTASVVCLLNNFYPREAKVQWKVDNALQSGNSQESVTEQDSKDSTYSLSSTLTLSKADYEKHKVYACEVTHQGLSSPVTKSFNRGEC

SEQ ID NO: 109 - protein, 448 aa, synthetic construct
  CHAIN 1..448: note = CH310-HC
EVQLQQSGPELVKPGASLKISCKASGYSFTGYYMNWVKQSPEKSLEWIGEINPSTGGSTYNQKFKAKATLTVDQSSNTAYMQLKSLTSEDSAVYYCARRELGGPFGYWGQGTPVTVSAASTKGPSVFPLAPSSKSTSGGTAALGCLVKDYFPEPVTVSWNSGALTSGVHTFPAVLQSSGLYSLSSVVTVPSSSLGTQTYICNVNHKPSNTKVDKKVEPKSCDKTHTCPPCPAPELLGGPSVFLFPPKPKDTLMISRTPEVTCVVVDVSHEDPEVKFNWYVDGVEVHNAKTKPREEQYNSTYRVVSVLTVLHQDWLNGKEYKCKVSNKALPAPIEKTISKAKGQPREPQVYTLPPSRDELTKNQVSLTCLVKGFYPSDIAVEWESNGQPENNYKTTPPVLDSDGSFFLYSKLTVDKSRWQQGNVFSCSVMHEALHNHYTQKSLSLSPGK

SEQ ID NO: 110 - protein, 214 aa, synthetic construct
  CHAIN 1..214: note = CH310-LC
SIVMTQTPKFLLVSSGDRVTITCKASQSVSNGIAWYQQKPGQSPKLLIYFASNRYTGVPDRFTGSGYGTDFTFTISTVQAEDLAVYFCQQDYSSPWTFGGGTKLEIKRTVAAPSVFIFPPSDEQLKSGTASVVCLLNNFYPREAKVQWKVDNALQSGNSQESVTEQDSKDSTYSLSSTLTLSKADYEKHKVYACEVTHQGLSSPVTKSFNRGEC

SEQ ID NO: 111 - protein, 11 aa, synthetic construct
  REGION 1..11: note = 310-VL6-LCDR1
KASQSVSQGIA

SEQ ID NO: 112 - protein, 11 aa, synthetic construct
  REGION 1..11: note = 310-VL7-LCDR1
KASQSVSSGIA

SEQ ID NO: 113 - protein, 11 aa, synthetic construct
  REGION 1..11: note = 310-VL8-LCDR1
KASQSVSTGIA

SEQ ID NO: 114 - protein, 118 aa, synthetic construct
  REGION 1..118: note = >hu310-VH2
EVQLVQSGAEVKKPGASVKVSCKASGYSFTGYYMNWVRQAPGQGLEWMGEINPSTGGSTYNQKFKARVTLTVDQSTNTAYMELSSLRSEDTAVYYCARRELGGPFGYWGQGTTVTVSS

SEQ ID NO: 115 - protein, 107 aa, synthetic construct
  REGION 1..107: note = >hu310-VL1
DIVMTQSPDSLAVSLGERATINCKASQSVSNGIAWYQQKPGQPPKLLIYFASNRYTGVPDRFSGSGSGTDFTLTISSLQAEDVAVYYCQQDYSSPWTFGGGTKVEIK

SEQ ID NO: 116 - protein, 107 aa, synthetic construct
  REGION 1..107: note = >hu310-VL3
SIVMTQSPKFLAVSLGERATINCKASQSVSNGIAWYQQKPGQSPKLLIYFASNRYTGVPDRFSGSGYGTDFTFTISSLQAEDVAVYYCQQDYSSPWTFGGGTKVEIK

SEQ ID NO: 117 - protein, 107 aa, synthetic construct
  REGION 1..107: note = >hu310-VL4
DIQMTQSPSSLSASVGDRVTITCKASQSVSNGIAWYQQKPGKAPKLLIYFASNRYTGVPSRFSGSGSGTDFTFTISSLQPEDIATYYCQQDYSSPWTFGGGTKVEIK

SEQ ID NO: 118 - protein, 107 aa, synthetic construct
  REGION 1..107: note = >hu310-VL5
SIQMTQSPSSLSASVGDRVTITCKASQSVSNGIAWYQQKPGKSPKLLIYFASNRYTGVPSRFSGSGYGTDFTFTISSLQPEDIATYYCQQDYSSPWTFGGGTKVEIK

SEQ ID NO: 119 - protein, 107 aa, synthetic construct
  REGION 1..107: note = >hu310-VL6
SIQMTQSPSSLSASVGDRVTITCKASQSVSQGIAWYQQKPGKSPKLLIYFASNRYTGVPSRFSGSGYGTDFTFTISSLQPEDIATYYCQQDYSSPWTFGGGTKVEIK

SEQ ID NO: 120 - protein, 107 aa, synthetic construct
  REGION 1..107: note = >hu310-VL7
SIQMTQSPSSLSASVGDRVTITCKASQSVSSGIAWYQQKPGKSPKLLIYFASNRYTGVPSRFSGSGYGTDFTFTISSLQPEDIATYYCQQDYSSPWTFGGGTKVEIK

SEQ ID NO: 121 - protein, 107 aa, synthetic construct
  REGION 1..107: note = >hu310-VL8
SIQMTQSPSSLSASVGDRVTITCKASQSVSTGIAWYQQKPGKSPKLLIYFASNRYTGVPSRFSGSGYGTDFTFTISSLQPEDIATYYCQQDYSSPWTFGGGTKVEIK

SEQ ID NO: 122 - protein, 448 aa, synthetic construct
  CHAIN 1..448: note = hu310-9/hu310-10/hu310-11/hu310-12/hu310-13/hu310-14/hu310-15/hu310-16-HC
EVQLVQSGAEVKKPGASVKVSCKASGYSFTGYYMNWVRQAPGQGLEWMGEINPSTGGSTYNQKFKARVTLTVDQSTNTAYMELSSLRSEDTAVYYCARRELGGPFGYWGQGTTVTVSSASTKGPSVFPLAPSSKSTSGGTAALGCLVKDYFPEPVTVSWNSGALTSGVHTFPAVLQSSGLYSLSSVVTVPSSSLGTQTYICNVNHKPSNTKVDKKVEPKSCDKTHTCPPCPAPELLGGPSVFLFPPKPKDTLMISRTPEVTCVVVDVSHEDPEVKFNWYVDGVEVHNAKTKPREEQYNSTYRVVSVLTVLHQDWLNGKEYKCKVSNKALPAPIEKTISKAKGQPREPQVYTLPPSRDELTKNQVSLTCLVKGFYPSDIAVEWESNGQPENNYKTTPPVLDSDGSFFLYSKLTVDKSRWQQGNVFSCSVMHEALHNHYTQKSLSLSPGK

SEQ ID NO: 123 - protein, 214 aa, synthetic construct
  CHAIN 1..214: note = hu310-1/hu310-9-LC
DIVMTQSPDSLAVSLGERATINCKASQSVSNGIAWYQQKPGQPPKLLIYFASNRYTGVPDRFSGSGSGTDFTLTISSLQAEDVAVYYCQQDYSSPWTFGGGTKVEIKRTVAAPSVFIFPPSDEQLKSGTASVVCLLNNFYPREAKVQWKVDNALQSGNSQESVTEQDSKDSTYSLSSTLTLSKADYEKHKVYACEVTHQGLSSPVTKSFNRGEC

SEQ ID NO: 124 - protein, 214 aa, synthetic construct
  CHAIN 1..214: note = hu310-3/hu310-11-LC
SIVMTQSPKFLAVSLGERATINCKASQSVSNGIAWYQQKPGQSPKLLIYFASNRYTGVPDRFSGSGYGTDFTFTISSLQAEDVAVYYCQQDYSSPWTFGGGTKVEIKRTVAAPSVFIFPPSDEQLKSGTASVVCLLNNFYPREAKVQWKVDNALQSGNSQESVTEQDSKDSTYSLSSTLTLSKADYEKHKVYACEVTHQGLSSPVTKSFNRGEC

SEQ ID NO: 125 - protein, 214 aa, synthetic construct
  CHAIN 1..214: note = hu310-4/hu310-12-LC
DIQMTQSPSSLSASVGDRVTITCKASQSVSNGIAWYQQKPGKAPKLLIYFASNRYTGVPSRFSGSGSGTDFTFTISSLQPEDIATYYCQQDYSSPWTFGGGTKVEIKRTVAAPSVFIFPPSDEQLKSGTASVVCLLNNFYPREAKVQWKVDNALQSGNSQESVTEQDSKDSTYSLSSTLTLSKADYEKHKVYACEVTHQGLSSPVTKSFNRGEC

SEQ ID NO: 126 - protein, 214 aa, synthetic construct
  CHAIN 1..214: note = hu310-5/hu310-13-LC
SIQMTQSPSSLSASVGDRVTITCKASQSVSNGIAWYQQKPGKSPKLLIYFASNRYTGVPSRFSGSGYGTDFTFTISSLQPEDIATYYCQQDYSSPWTFGGGTKVEIKRTVAAPSVFIFPPSDEQLKSGTASVVCLLNNFYPREAKVQWKVDNALQSGNSQESVTEQDSKDSTYSLSSTLTLSKADYEKHKVYACEVTHQGLSSPVTKSFNRGEC

SEQ ID NO: 127 - protein, 214 aa, synthetic construct
  CHAIN 1..214: note = hu310-6/hu310-14-LC
SIQMTQSPSSLSASVGDRVTITCKASQSVSQGIAWYQQKPGKSPKLLIYFASNRYTGVPSRFSGSGYGTDFTFTISSLQPEDIATYYCQQDYSSPWTFGGGTKVEIKRTVAAPSVFIFPPSDEQLKSGTASVVCLLNNFYPREAKVQWKVDNALQSGNSQESVTEQDSKDSTYSLSSTLTLSKADYEKHKVYACEVTHQGLSSPVTKSFNRGEC

SEQ ID NO: 128 - protein, 214 aa, synthetic construct
  CHAIN 1..214: note = hu310-7/hu310-15-LC
SIQMTQSPSSLSASVGDRVTITCKASQSVSSGIAWYQQKPGKSPKLLIYFASNRYTGVPSRFSGSGYGTDFTFTISSLQPEDIATYYCQQDYSSPWTFGGGTKVEIKRTVAAPSVFIFPPSDEQLKSGTASVVCLLNNFYPREAKVQWKVDNALQSGNSQESVTEQDSKDSTYSLSSTLTLSKADYEKHKVYACEVTHQGLSSPVTKSFNRGEC

SEQ ID NO: 129 - protein, 214 aa, synthetic construct
  CHAIN 1..214: note = hu310-8/hu310-16-LC
SIQMTQSPSSLSASVGDRVTITCKASQSVSTGIAWYQQKPGKSPKLLIYFASNRYTGVPSRFSGSGYGTDFTFTISSLQPEDIATYYCQQDYSSPWTFGGGTKVEIKRTVAAPSVFIFPPSDEQLKSGTASVVCLLNNFYPREAKVQWKVDNALQSGNSQESVTEQDSKDSTYSLSSTLTLSKADYEKHKVYACEVTHQGLSSPVTKSFNRGEC

SEQ ID NO: 130 - protein, 120 aa, synthetic construct
  REGION 1..120: note = >hu67-VH1
EVTLKQSGPVLVKPTQTLTLTCTVSGFSLTNYGVNWIRQPPRKALEWLAVIWSRGNTDYNAAFISRLTISKDTSKSQVVLKMTNMDPVDTATYYCARKDAVVATDALDYWGQGTTVTVSS

SEQ ID NO: 131 - protein, 120 aa, synthetic construct
  REGION 1..120: note = >hu67-VH2
EVTLKQSGPVLVKPTQTLTLTCTVSGFSLTNYGVNWIRQPPRKGLEWLGVIWSRGNTDYNAAFISRLTISKDNSKSQVVLKMTNMDPVDTATYYCARKDAVVATDALDYWGQGTTVTVSS

SEQ ID NO: 132 - protein, 120 aa, synthetic construct
  REGION 1..120: note = >hu67-VH4
EVQLQESGPGLVKPSQTLSLTCTVSGFSLTNYGVNWIRQPPRKGLEWIGVIWSRGNTDYNAAFISRVTISKDNSKSQVSLKLSSVTAADTAVYYCARKDAVVATDALDYWGQGTTVTVSS

SEQ ID NO: 133 - protein, 107 aa, synthetic construct
  REGION 1..107: note = >67VL-VL1
DIVMTQSPKSLAVSLGERATINCKASQDVSTAVAWYQQKPGQPPKLLIYSTSYRYTGVPDRFSGSGSGTDFTLTISSLQAEDVAVYYCQQHYSTPYTFGGGTKVEIK

SEQ ID NO: 134 - protein, 107 aa, synthetic construct
  REGION 1..107: note = >67VL-VL2
DIVMTQSPKSLAVSLGERATINCKASQDVSTAVAWYQQKPGQSPKLLIYSTSYRYTGVPDRFSGSGSGTDFTFTISSLQAEDVAVYYCQQHYSTPYTFGGGTKVEIK

SEQ ID NO: 135 - protein, 107 aa, synthetic construct
  REGION 1..107: note = >67VL-VL4
DIQMTQSHKFLSASVGDRVTITCKASQDVSTAVAWYQQKPGKSPKLLIYSTSYRYTGVPSRFSGSGSGTDFTFTISSLQPEDIATYYCQQHYSTPYTFGGGTKVEIK

SEQ ID NO: 136 - protein, 450 aa, synthetic construct
  CHAIN 1..450: note = hu67-1/hu67-5/hu67-9/hu67-13-HC
EVTLKQSGPVLVKPTQTLTLTCTVSGFSLTNYGVNWIRQPPRKALEWLAVIWSRGNTDYNAAFISRLTISKDTSKSQVVLKMTNMDPVDTATYYCARKDAVVATDALDYWGQGTTVTVSSASTKGPSVFPLAPSSKSTSGGTAALGCLVKDYFPEPVTVSWNSGALTSGVHTFPAVLQSSGLYSLSSVVTVPSSSLGTQTYICNVNHKPSNTKVDKKVEPKSCDKTHTCPPCPAPELLGGPSVFLFPPKPKDTLMISRTPEVTCVVVDVSHEDPEVKFNWYVDGVEVHNAKTKPREEQYNSTYRVVSVLTVLHQDWLNGKEYKCKVSNKALPAPIEKTISKAKGQPREPQVYTLPPSRDELTKNQVSLTCLVKGFYPSDIAVEWESNGQPENNYKTTPPVLDSDGSFFLYSKLTVDKSRWQQGNVFSCSVMHEALHNHYTQKSLSLSPGK

SEQ ID NO: 137 - protein, 450 aa, synthetic construct
  CHAIN 1..450: note = hu67-2/hu67-6/hu67-10/hu67-14-HC
EVTLKQSGPVLVKPTQTLTLTCTVSGFSLTNYGVNWIRQPPRKGLEWLGVIWSRGNTDYNAAFISRLTISKDNSKSQVVLKMTNMDPVDTATYYCARKDAVVATDALDYWGQGTTVTVSSASTKGPSVFPLAPSSKSTSGGTAALGCLVKDYFPEPVTVSWNSGALTSGVHTFPAVLQSSGLYSLSSVVTVPSSSLGTQTYICNVNHKPSNTKVDKKVEPKSCDKTHTCPPCPAPELLGGPSVFLFPPKPKDTLMISRTPEVTCVVVDVSHEDPEVKFNWYVDGVEVHNAKTKPREEQYNSTYRVVSVLTVLHQDWLNGKEYKCKVSNKALPAPIEKTISKAKGQPREPQVYTLPPSRDELTKNQVSLTCLVKGFYPSDIAVEWESNGQPENNYKTTPPVLDSDGSFFLYSKLTVDKSRWQQGNVFSCSVMHEALHNHYTQKSLSLSPGK

SEQ ID NO: 138 - protein, 450 aa, synthetic construct
  CHAIN 1..450: note = hu67-4/hu67-8/hu67-12/hu67-16-HC
EVQLQESGPGLVKPSQTLSLTCTVSGFSLTNYGVNWIRQPPRKGLEWIGVIWSRGNTDYNAAFISRVTISKDNSKSQVSLKLSSVTAADTAVYYCARKDAVVATDALDYWGQGTTVTVSSASTKGPSVFPLAPSSKSTSGGTAALGCLVKDYFPEPVTVSWNSGALTSGVHTFPAVLQSSGLYSLSSVVTVPSSSLGTQTYICNVNHKPSNTKVDKKVEPKSCDKTHTCPPCPAPELLGGPSVFLFPPKPKDTLMISRTPEVTCVVVDVSHEDPEVKFNWYVDGVEVHNAKTKPREEQYNSTYRVVSVLTVLHQDWLNGKEYKCKVSNKALPAPIEKTISKAKGQPREPQVYTLPPSRDELTKNQVSLTCLVKGFYPSDIAVEWESNGQPENNYKTTPPVLDSDGSFFLYSKLTVDKSRWQQGNVFSCSVMHEALHNHYTQKSLSLSPGK

SEQ ID NO: 139 - protein, 214 aa, synthetic construct
  CHAIN 1..214: note = hu67-1/hu67-2/hu67-3/hu67-4-LC
DIVMTQSPKSLAVSLGERATINCKASQDVSTAVAWYQQKPGQPPKLLIYSTSYRYTGVPDRFSGSGSGTDFTLTISSLQAEDVAVYYCQQHYSTPYTFGGGTKVEIKRTVAAPSVFIFPPSDEQLKSGTASVVCLLNNFYPREAKVQWKVDNALQSGNSQESVTEQDSKDSTYSLSSTLTLSKADYEKHKVYACEVTHQGLSSPVTKSFNRGEC

SEQ ID NO: 140 - protein, 214 aa, synthetic construct
  CHAIN 1..214: note = hu67-5/hu67-6/hu67-7/hu67-8-LC
DIVMTQSPKSLAVSLGERATINCKASQDVSTAVAWYQQKPGQSPKLLIYSTSYRYTGVPDRFSGSGSGTDFTFTISSLQAEDVAVYYCQQHYSTPYTFGGGTKVEIKRTVAAPSVFIFPPSDEQLKSGTASVVCLLNNFYPREAKVQWKVDNALQSGNSQESVTEQDSKDSTYSLSSTLTLSKADYEKHKVYACEVTHQGLSSPVTKSFNRGEC

SEQ ID NO: 141 - protein, 214 aa, synthetic construct
  CHAIN 1..214: note = hu67-13/hu67-14/hu67-15/hu67-16-LC
DIQMTQSHKFLSASVGDRVTITCKASQDVSTAVAWYQQKPGKSPKLLIYSTSYRYTGVPSRFSGSGSGTDFTFTISSLQPEDIATYYCQQHYSTPYTFGGGTKVEIKRTVAAPSVFIFPPSDEQLKSGTASVVCLLNNFYPREAKVQWKVDNALQSGNSQESVTEQDSKDSTYSLSSTLTLSKADYEKHKVYACEVTHQGLSSPVTKSFNRGEC

SEQ ID NO: 142 - protein, 17 aa, synthetic construct
  REGION 1..17: note = hu10H10VH5-HCDR2
DILPGSGSSNYNENFKG

SEQ ID NO: 143 - protein, 11 aa, synthetic construct
  REGION 1..11: note = hu10H10VH6-HCDR3
SGYYGNSGFVY

SEQ ID NO: 144 - protein, 5 aa, synthetic construct
  REGION 1..5: note = hu10H10VH10-HCDR1
EYWIE

SEQ ID NO: 145 - protein, 17 aa, synthetic construct
  REGION 1..17: note = hu10H10VH12-HCDR2
DILPGHGSTNYNENFKG

SEQ ID NO: 146 - protein, 17 aa, synthetic construct
  REGION 1..17: note = hu10H10VH13/VH14-HCDR2
DILPGSGWTNYNENFKG

SEQ ID NO: 147 - protein, 17 aa, synthetic construct
  REGION 1..17: note = hu10H10VL2-LCDR1
RASQSILSSGNQKNYLT

SEQ ID NO: 148 - protein, 7 aa, synthetic construct
  REGION 1..7: note = hu10H10VL3/VL5/VL6-LCDR2
WASTREE

SEQ ID NO: 149 - protein, 9 aa, synthetic construct
  REGION 1..9: note = hu10H10VL4-LCDR3
QNDYTYPLS

SEQ ID NO: 150 - protein, 17 aa, synthetic construct
  REGION 1..17: note = hu10H10VL5-LCDR1
KSSQSLLDSGNQKNYLT

SEQ ID NO: 151 - protein, 17 aa, synthetic construct
  REGION 1..17: note = hu10H10VL6-LCDR1
KSSQSLLSSSNQKNYLT

SEQ ID NO: 152 - protein, 450 aa, synthetic construct
  CHAIN 1..450: note = hu10H10-1/hu10H10-7/hu10H10-13/hu10H10-19-HC
EVQLVQSGAEVKKPGASVKVSCKASGYTFITYWIEWVRQRPGQGLEWMGDILPGSGSTNYNENFKGRVTFTADTSTSTVYMQLSSLRSEDTAVYYCARSGYYGNSGFAYWGQGTLVTVSSASTKGPSVFPLAPSSKSTSGGTAALGCLVKDYFPEPVTVSWNSGALTSGVHTFPAVLQSSGLYSLSSVVTVPSSSLGTQTYICNVNHKPSNTKVDKKVEPKSCDKTHTCPPCPAPELLGGPSVFLFPPKPKDTLMISRTPEVTCVVVDVSHEDPEVKFNWYVDGVEVHNAKTKPREEQYNSTYRVVSVLTVLHQDWLNGKEYKCKVSNKALPAPIEKTISKAKGQPREPQVYTLPPSRDELTKNQVSLTCLVKGFYPSDIAVEWESNGQPENNYKTTPPVLDSDGSFFLYSKLTVDKSRWQQGNVFSCSVMHEALHNHYTQKSLSLSPGK

SEQ ID NO: 153 - protein, 450 aa, synthetic construct
  CHAIN 1..450: note = hu10H10-2/hu10H10-8/hu10H10-14/hu10H10-20/hu10H10-57/hu10H10-58-HC
EVQLVQSGSELKKPGASVKVSCKASGYTFITYWIEWVRQRPGQGLEWMGDILPGSGSTNYNENFKGRAVFSADTSVSTAYLQISSLKAEDTAVYYCARSGYYGNSGFAYWGQGTLVTVSSASTKGPSVFPLAPSSKSTSGGTAALGCLVKDYFPEPVTVSWNSGALTSGVHTFPAVLQSSGLYSLSSVVTVPSSSLGTQTYICNVNHKPSNTKVDKKVEPKSCDKTHTCPPCPAPELLGGPSVFLFPPKPKDTLMISRTPEVTCVVVDVSHEDPEVKFNWYVDGVEVHNAKTKPREEQYNSTYRVVSVLTVLHQDWLNGKEYKCKVSNKALPAPIEKTISKAKGQPREPQVYTLPPSRDELTKNQVSLTCLVKGFYPSDIAVEWESNGQPENNYKTTPPVLDSDGSFFLYSKLTVDKSRWQQGNVFSCSVMHEALHNHYTQKSLSLSPGK

SEQ ID NO: 154 - protein, 450 aa, synthetic construct
  CHAIN 1..450: note = hu10H10-3/hu10H10-9/hu10H10-15/hu10H10-21-HC
EVQLVQSGAEVKKPGASVKVSCKASIYTFITYWIEWVRQRPGQGLEWMGDILPGSGSTNYNENFKGRVTFTADTSTSTVYMQLSSLRSEDTAVYYCARSGYYGNSGFAYWGQGTLVTVSSASTKGPSVFPLAPSSKSTSGGTAALGCLVKDYFPEPVTVSWNSGALTSGVHTFPAVLQSSGLYSLSSVVTVPSSSLGTQTYICNVNHKPSNTKVDKKVEPKSCDKTHTCPPCPAPELLGGPSVFLFPPKPKDTLMISRTPEVTCVVVDVSHEDPEVKFNWYVDGVEVHNAKTKPREEQYNSTYRVVSVLTVLHQDWLNGKEYKCKVSNKALPAPIEKTISKAKGQPREPQVYTLPPSRDELTKNQVSLTCLVKGFYPSDIAVEWESNGQPENNYKTTPPVLDSDGSFFLYSKLTVDKSRWQQGNVFSCSVMHEALHNHYTQKSLSLSPGK

SEQ ID NO: 155 - protein, 450 aa, synthetic construct
  CHAIN 1..450: note = hu10H10-4/hu10H10-10/hu10H10-16/hu10H10-22-HC
EVQLVQSGSELKKPGASVKVSCKASGFTFITYWIEWVRQRPGQGLEWMGDILPGSGSTNYNENFKGRAVFSADTSVSTAYLQISSLKAEDTAVYYCARSGYYGNSGFAYWGQGTLVTVSSASTKGPSVFPLAPSSKSTSGGTAALGCLVKDYFPEPVTVSWNSGALTSGVHTFPAVLQSSGLYSLSSVVTVPSSSLGTQTYICNVNHKPSNTKVDKKVEPKSCDKTHTCPPCPAPELLGGPSVFLFPPKPKDTLMISRTPEVTCVVVDVSHEDPEVKFNWYVDGVEVHNAKTKPREEQYNSTYRVVSVLTVLHQDWLNGKEYKCKVSNKALPAPIEKTISKAKGQPREPQVYTLPPSRDELTKNQVSLTCLVKGFYPSDIAVEWESNGQPENNYKTTPPVLDSDGSFFLYSKLTVDKSRWQQGNVFSCSVMHEALHNHYTQKSLSLSPGK

SEQ ID NO: 156 - protein, 450 aa, synthetic construct
  CHAIN 1..450: note = hu10H10-5/hu10H10-11/hu10H10-17/hu10H10-23-HC
EVQLVQSGAEVKKPGASVKVSCKASGYTFITYWIEWVRQRPGQGLEWMGDILPGSGSSNYNENFKGRVTFTADTSTSTVYMQLSSLRSEDTAVYYCARSGYYGNSGFAYWGQGTLVTVSSASTKGPSVFPLAPSSKSTSGGTAALGCLVKDYFPEPVTVSWNSGALTSGVHTFPAVLQSSGLYSLSSVVTVPSSSLGTQTYICNVNHKPSNTKVDKKVEPKSCDKTHTCPPCPAPELLGGPSVFLFPPKPKDTLMISRTPEVTCVVVDVSHEDPEVKFNWYVDGVEVHNAKTKPREEQYNSTYRVVSVLTVLHQDWLNGKEYKCKVSNKALPAPIEKTISKAKGQPREPQVYTLPPSRDELTKNQVSLTCLVKGFYPSDIAVEWESNGQPENNYKTTPPVLDSDGSFFLYSKLTVDKSRWQQGNVFSCSVMHEALHNHYTQKSLSLSPGK

SEQ ID NO: 157 - protein, 450 aa, synthetic construct
  CHAIN 1..450: note = hu10H10-6/hu10H10-12/hu10H10-18/hu10H10-24-HC
EVQLVQSGSELKKPGASVKVSCKASGYTFITYWIEWVRQRPGQGLEWMGDILPGSGSTNYNENFKGRAVFSADTSVSTAYLQISSLKAEDTAVYYCARSGYYGNSGFVYWGQGTLVTVSSASTKGPSVFPLAPSSKSTSGGTAALGCLVKDYFPEPVTVSWNSGALTSGVHTFPAVLQSSGLYSLSSVVTVPSSSLGTQTYICNVNHKPSNTKVDKKVEPKSCDKTHTCPPCPAPELLGGPSVFLFPPKPKDTLMISRTPEVTCVVVDVSHEDPEVKFNWYVDGVEVHNAKTKPREEQYNSTYRVVSVLTVLHQDWLNGKEYKCKVSNKALPAPIEKTISKAKGQPREPQVYTLPPSRDELTKNQVSLTCLVKGFYPSDIAVEWESNGQPENNYKTTPPVLDSDGSFFLYSKLTVDKSRWQQGNVFSCSVMHEALHNHYTQKSLSLSPGK

SEQ ID NO: 158 - protein, 450 aa, synthetic construct
  CHAIN 1..450: note = hu10H10-25/hu10H10-33/hu10H10-41/hu10H10-49-HC
EVQLVQSGSELKKPGASVKVSCKASGYTFITYWIEWVKQRPGQGLEWMGDILPGSGSTNYNENFKGRATFSADTSVSTAYLQISSLKAEDTAVYYCARSGYYGNSGFAYWGQGTLVTVSSASTKGPSVFPLAPSSKSTSGGTAALGCLVKDYFPEPVTVSWNSGALTSGVHTFPAVLQSSGLYSLSSVVTVPSSSLGTQTYICNVNHKPSNTKVDKKVEPKSCDKTHTCPPCPAPELLGGPSVFLFPPKPKDTLMISRTPEVTCVVVDVSHEDPEVKFNWYVDGVEVHNAKTKPREEQYNSTYRVVSVLTVLHQDWLNGKEYKCKVSNKALPAPIEKTISKAKGQPREPQVYTLPPSRDELTKNQVSLTCLVKGFYPSDIAVEWESNGQPENNYKTTPPVLDSDGSFFLYSKLTVDKSRWQQGNVFSCSVMHEALHNHYTQKSLSLSPGK

SEQ ID NO: 159 - protein, 450 aa, synthetic construct
  CHAIN 1..450: note = hu10H10-26/hu10H10-34/hu10H10-42/hu10H10-50-HC
EVQLVQSGSELKKPGASVKVSCKASGRTFITYWIEWVRQRPGQGLEWMGDILPGSGSTNYNENFKGRATFSADTSVSTAYLQISSLKAEDTAVYYCARSGYYGNSGFAYWGQGTLVTVSSASTKGPSVFPLAPSSKSTSGGTAALGCLVKDYFPEPVTVSWNSGALTSGVHTFPAVLQSSGLYSLSSVVTVPSSSLGTQTYICNVNHKPSNTKVDKKVEPKSCDKTHTCPPCPAPELLGGPSVFLFPPKPKDTLMISRTPEVTCVVVDVSHEDPEVKFNWYVDGVEVHNAKTKPREEQYNSTYRVVSVLTVLHQDWLNGKEYKCKVSNKALPAPIEKTISKAKGQPREPQVYTLPPSRDELTKNQVSLTCLVKGFYPSDIAVEWESNGQPENNYKTTPPVLDSDGSFFLYSKLTVDKSRWQQGNVFSCSVMHEALHNHYTQKSLSLSPGK

SEQ ID NO: 160 - protein, 450 aa, synthetic construct
  CHAIN 1..450: note = hu10H10-27/hu10H10-35/hu10H10-43/hu10H10-51-HC
EVQLVQSGSELKKPGASVKVSCKASGYTFRTYWIEWVKQRPGQGLEWMGDILPGSGSTNYNENFKGRATFSADTSVSTAYLQISSLKAEDTAVYYCARSGYYGNSGFAYWGQGTLVTVSSASTKGPSVFPLAPSSKSTSGGTAALGCLVKDYFPEPVTVSWNSGALTSGVHTFPAVLQSSGLYSLSSVVTVPSSSLGTQTYICNVNHKPSNTKVDKKVEPKSCDKTHTCPPCPAPELLGGPSVFLFPPKPKDTLMISRTPEVTCVVVDVSHEDPEVKFNWYVDGVEVHNAKTKPREEQYNSTYRVVSVLTVLHQDWLNGKEYKCKVSNKALPAPIEKTISKAKGQPREPQVYTLPPSRDELTKNQVSLTCLVKGFYPSDIAVEWESNGQPENNYKTTPPVLDSDGSFFLYSKLTVDKSRWQQGNVFSCSVMHEALHNHYTQKSLSLSPGK

SEQ ID NO: 161 - protein, 450 aa, synthetic construct
  CHAIN 1..450: note = hu10H10-28/hu10H10-36/hu10H10-44/hu10H10-52-HC
EVQLVQSGSELKKPGASVKVSCKASGYTFIEYWIEWVKQRPGQGLEWMGDILPGSGSTNYNENFKGRATFSADTSVSTAYLQISSLKAEDTAVYYCARSGYYGNSGFAYWGQGTLVTVSSASTKGPSVFPLAPSSKSTSGGTAALGCLVKDYFPEPVTVSWNSGALTSGVHTFPAVLQSSGLYSLSSVVTVPSSSLGTQTYICNVNHKPSNTKVDKKVEPKSCDKTHTCPPCPAPELLGGPSVFLFPPKPKDTLMISRTPEVTCVVVDVSHEDPEVKFNWYVDGVEVHNAKTKPREEQYNSTYRVVSVLTVLHQDWLNGKEYKCKVSNKALPAPIEKTISKAKGQPREPQVYTLPPSRDELTKNQVSLTCLVKGFYPSDIAVEWESNGQPENNYKTTPPVLDSDGSFFLYSKLTVDKSRWQQGNVFSCSVMHEALHNHYTQKSLSLSPGK

SEQ ID NO: 162 - protein, 450 aa, synthetic construct
  CHAIN 1..450: note = hu10H10-30/hu10H10-38/hu10H10-46/hu10H10-54-HC
EVQLVQSGSELKKPGASVKVSCKASGYTFITYWIEWVKQRPGQGLEWMGDILPGHGSTNYNENFKGRATFSADTSVSTAYLQISSLKAEDTAVYYCARSGYYGNSGFAYWGQGTLVTVSSASTKGPSVFPLAPSSKSTSGGTAALGCLVKDYFPEPVTVSWNSGALTSGVHTFPAVLQSSGLYSLSSVVTVPSSSLGTQTYICNVNHKPSNTKVDKKVEPKSCDKTHTCPPCPAPELLGGPSVFLFPPKPKDTLMISRTPEVTCVVVDVSHEDPEVKFNWYVDGVEVHNAKTKPREEQYNSTYRVVSVLTVLHQDWLNGKEYKCKVSNKALPAPIEKTISKAKGQPREPQVYTLPPSRDELTKNQVSLTCLVKGFYPSDIAVEWESNGQPENNYKTTPPVLDSDGSFFLYSKLTVDKSRWQQGNVFSCSVMHEALHNHYTQKSLSLSPGK

SEQ ID NO: 163 - protein, 450 aa, synthetic construct
  CHAIN 1..450: note = hu10H10-31/hu10H10-39/hu10H10-47/hu10H10-55-HC
EVQLVQSGSELKKPGASVKVSCKASGYTFITYWIEWVKQRPGQGLEWMGDILPGSGWTNYNENFKGRATFSADTSVSTAYLQISSLKAEDTAVYYCARSGYYGNSGFAYWGQGTLVTVSSASTKGPSVFPLAPSSKSTSGGTAALGCLVKDYFPEPVTVSWNSGALTSGVHTFPAVLQSSGLYSLSSVVTVPSSSLGTQTYICNVNHKPSNTKVDKKVEPKSCDKTHTCPPCPAPELLGGPSVFLFPPKPKDTLMISRTPEVTCVVVDVSHEDPEVKFNWYVDGVEVHNAKTKPREEQYNSTYRVVSVLTVLHQDWLNGKEYKCKVSNKALPAPIEKTISKAKGQPREPQVYTLPPSRDELTKNQVSLTCLVKGFYPSDIAVEWESNGQPENNYKTTPPVLDSDGSFFLYSKLTVDKSRWQQGNVFSCSVMHEALHNHYTQKSLSLSPGK

SEQ ID NO: 164 - protein, 450 aa, synthetic construct
  CHAIN 1..450: note = hu10H10-32/hu10H10-40/hu10H10-48/hu10H10-56-HC
EVQLVQSGSELKKPGASVKVSCKASGYTFITYWIEWVRQRPGQGLEWMGDILPGSGWTNYNENFKGRAVFSADTSVSTAYLQISSLKAEDTAVYYCARSGYYGNSGFAYWGQGTLVTVSSASTKGPSVFPLAPSSKSTSGGTAALGCLVKDYFPEPVTVSWNSGALTSGVHTFPAVLQSSGLYSLSSVVTVPSSSLGTQTYICNVNHKPSNTKVDKKVEPKSCDKTHTCPPCPAPELLGGPSVFLFPPKPKDTLMISRTPEVTCVVVDVSHEDPEVKFNWYVDGVEVHNAKTKPREEQYNSTYRVVSVLTVLHQDWLNGKEYKCKVSNKALPAPIEKTISKAKGQPREPQVYTLPPSRDELTKNQVSLTCLVKGFYPSDIAVEWESNGQPENNYKTTPPVLDSDGSFFLYSKLTVDKSRWQQGNVFSCSVMHEALHNHYTQKSLSLSPGK

SEQ ID NO: 165 - protein, 220 aa, synthetic construct
  CHAIN 1..220: note = hu10H10-1/hu10H10-2/hu10H10-3/hu10H10-4/hu10H10-5/hu10H10-6/hu10H10-25/hu10H10-26/hu10H10-27/hu10H10-28/hu10H10-29/hu10H10-30/hu10H10-31/hu10H10-32-LC
DIQMTQSPSSLSASVGDRVTITCKSSQSLLSSGNQKNYLTWYQQKPGKAPKLLIYWASTRESGVPSRFSGSGSGTDFTLTISSLQPEDFATYYCQNDYTYPLTFGQGTKLEIKRTVAAPSVFIFPPSDEQLKSGTASVVCLLNNFYPREAKVQWKVDNALQSGNSQESVTEQDSKDSTYSLSSTLTLSKADYEKHKVYACEVTHQGLSSPVTKSFNRGEC

SEQ ID NO: 166 - protein, 220 aa, synthetic construct
  CHAIN 1..220: note = hu10H10-7/hu10H10-8/hu10H10-9/hu10H10-10/hu10H10-11/hu10H10-12-LC
DIQMTQSPSSLSASVGDRVTITCRASQSILSSGNQKNYLTWYQQKPGKAPKLLIYWASTRESGVPSRFSGSGSGTDFTLTISSLQPEDFATYYCQNDYTYPLTFGQGTKLEIKRTVAAPSVFIFPPSDEQLKSGTASVVCLLNNFYPREAKVQWKVDNALQSGNSQESVTEQDSKDSTYSLSSTLTLSKADYEKHKVYACEVTHQGLSSPVTKSFNRGEC

SEQ ID NO: 167 - protein, 220 aa, synthetic construct
  CHAIN 1..220: note = hu10H10-13/hu10H10-14/hu10H10-15/hu10H10-16/hu10H10-17/hu10H10-18/hu10H10-33/hu10H10-34/hu10H10-35/hu10H10-36/hu10H10-37/hu10H10-38/hu10H10-39/hu10H10-40-LC
DIQMTQSPSSLSASVGDRVTITCKSSQSLLSSGNQKNYLTWYQQKPGKAPKLLIYWASTREEGVPSRFSGSGSGTDFTLTISSLQPEDFATYYCQNDYTYPLTFGQGTKLEIKRTVAAPSVFIFPPSDEQLKSGTASVVCLLNNFYPREAKVQWKVDNALQSGNSQESVTEQDSKDSTYSLSSTLTLSKADYEKHKVYACEVTHQGLSSPVTKSFNRGEC

SEQ ID NO: 168 - protein, 220 aa, synthetic construct
  CHAIN 1..220: note = hu10H10-19/hu10H10-20/hu10H10-21/hu10H10-22/hu10H10-23/hu10H10-24-LC
DIQMTQSPSSLSASVGDRVTITCKSSQSLLSSGNQKNYLTWYQQKPGKAPKLLIYWASTRESGVPSRFSGSGSGTDFTLTISSLQPEDFATYYCQNDYTYPLSFGQGTKLEIKRTVAAPSVFIFPPSDEQLKSGTASVVCLLNNFYPREAKVQWKVDNALQSGNSQESVTEQDSKDSTYSLSSTLTLSKADYEKHKVYACEVTHQGLSSPVTKSFNRGEC

SEQ ID NO: 169 - protein, 220 aa, synthetic construct
  CHAIN 1..220: note = hu10H10-41/hu10H10-42/hu10H10-43/hu10H10-44/hu10H10-45/hu10H10-46/hu10H10-47/hu10H10-48/hu10H10-57-LC
DIQMTQSPSSLSASVGDRVTITCKSSQSLLDSGNQKNYLTWYQQKPGKAPKLLIYWASTREEGVPSRFSGSGSGTDFTLTISSLQPEDFATYYCQNDYTYPLTFGQGTKLEIKRTVAAPSVFIFPPSDEQLKSGTASVVCLLNNFYPREAKVQWKVDNALQSGNSQESVTEQDSKDSTYSLSSTLTLSKADYEKHKVYACEVTHQGLSSPVTKSFNRGEC

SEQ ID NO: 170 - protein, 220 aa, synthetic construct
  CHAIN 1..220: note = hu10H10-49/hu10H10-50/hu10H10-51/hu10H10-52/hu10H10-53/hu10H10-54/hu10H10-55/hu10H10-56/hu10H10-58-LC
DIQMTQSPSSLSASVGDRVTITCKSSQSLLSSSNQKNYLTWYQQKPGKAPKLLIYWASTREEGVPSRFSGSGSGTDFTLTISSLQPEDFATYYCQNDYTYPLTFGQGTKLEIKRTVAAPSVFIFPPSDEQLKSGTASVVCLLNNFYPREAKVQWKVDNALQSGNSQESVTEQDSKDSTYSLSSTLTLSKADYEKHKVYACEVTHQGLSSPVTKSFNRGEC

SEQ ID NO: 171 - protein, 242 aa, synthetic construct
  CHAIN 1..242: note = hu67-11-scFv
EVQLQESGPGLVKPSQTLSLTCTVSGFSLTNYGVNWIRQPPGKGLEWIGVIWSRGNTDYNAAFISRVTISKDTSKNQVSLKLSSVTAADTAVYYCARKDAVVATDALDYWGQGTTVTVSSGGGGSGGGGSGGGGSDIQMTQSPSSLSASVGDRVTITCKASQDVSTAVAWYQQKPGKAPKLLIYSTSYRYTGVPSRFSGSGSGTDFTFTISSLQPEDIATYYCQQHYSTPYTFGGGTKVEIK